European Patent Application EP 4 183 406 A1, published May 24, 2023. Title: IN VITRO METHODS AND KITS FOR RESPIRATORY TRACT VIRAL DISEASES. Applicant: Fundación para el Fomento de la Investigación Sanitaria y Biomédica de la Comunitat Valenciana (FISABIO). The sequence listing filed with the application follows.

SEQUENCE LISTING (31 sequences)

SEQ ID NO: 1 - protein, 42 aa, Homo sapiens
  LEK-42
LEKGLDGAKKAVGGLGKLGKDAVEDLESVGKGAVHDVKDVLD

SEQ ID NO: 2 - protein, 45 aa, Homo sapiens
  LEK-45
LEKGLDGAKKAVGGLGKLGKDAVEDLESVGKGAVHDVKDVLDSVL

SEQ ID NO: 3 - protein, 45 aa, Homo sapiens
  SSL-45
SSLLEKGLDGAKKAVGGLGKLGKDAVEDLESVGKGAVHDVKDVLD

SEQ ID NO: 4 - protein, 47 aa, Homo sapiens
  DCD
SSLLEKGLDGAKKAVGGLGKLGKDAVEDLESVGKGAVHDVKDVLDSV

SEQ ID NO: 5 - protein, 48 aa, Homo sapiens
  DCD-1L
SSLLEKGLDGAKKAVGGLGKLGKDAVEDLESVGKGAVHDVKDVLDSVL

SEQ ID NO: 6 - protein, 46 aa, Homo sapiens
  SSL-46
SSLLEKGLDGAKKAVGGLGKLGKDAVEDLESVGKGAVHDVKDVLDS

SEQ ID NO: 7 - protein, 44 aa, Homo sapiens
  LEK-44
LEKGLDGAKKAVGGLGKLGKDAVEDLESVGKGAVHDVKDVLDSV

SEQ ID NO: 8 - protein, 43 aa, Homo sapiens
  LEK-43
LEKGLDGAKKAVGGLGKLGKDAVEDLESVGKGAVHDVKDVLDS

SEQ ID NO: 9 - protein, 29 aa, Homo sapiens
  SSL-29
SSLLEKGLDGAKKAVGGLGKLGKDAVEDL

SEQ ID NO: 10 - protein, 25 aa, Homo sapiens
  SSL-25
SSLLEKGLDGAKKAVGGLGKLGKDA

SEQ ID NO: 11 - protein, 41 aa, Homo sapiens
  LEK-41
LEKGLDGAKKAVGGLGKLGKDAVEDLESVGKGAVHDVKDVL

SEQ ID NO: 12 - protein, 26 aa, Homo sapiens
  LEK-26
LEKGLDGAKKAVGGLGKLGKDAVEDL

SEQ ID NO: 13 - protein, 24 aa, Homo sapiens
  LEK-24
LEKGLDGAKKAVGGLGKLGKDAVE

SEQ ID NO: 14 - protein, 42 aa, Homo sapiens
  YDP-42
YDPEAASAPGSGNPCHEASAAQKENAGEDPGLARQAPKPRKQ

SEQ ID NO: 15 - protein, 30 aa, Homo sapiens
  Y-P30
YDPEAASAPGSGNPCHEASAAQKENAGEDP

SEQ ID NO: 16 - protein, 20 aa, Homo sapiens
  PIF
YDPEAASAPGSGNPCHEASA

SEQ ID NO: 17 - protein, 110 aa, Homo sapiens
  Dermcidin
MRFMTLLFLTALAGALVCAYDPEAASAPGSGNPCHEASAAQKENAGEDPGLARQAPKPRKQRSSLLEKGLDGAKKAVGGLGKLGKDAVEDLESVGKGAVHDVKDVLDSVL

SEQ ID NO: 18 - protein, 42 aa, Homo sapiens; identical to SEQ ID NO: 1
  LEK-42
  MOD_RES 3: ACETYLATION

SEQ ID NO: 19 - protein, 45 aa, Homo sapiens; identical to SEQ ID NO: 2
  LEK-45
  MOD_RES 3: ACETYLATION

SEQ ID NO: 20 - protein, 45 aa, Homo sapiens; identical to SEQ ID NO: 3
  SSL-45
  MOD_RES 6: ACETYLATION

SEQ ID NO: 21 - protein, 47 aa, Homo sapiens; identical to SEQ ID NO: 4
  DCD
  MOD_RES 6: ACETYLATION

SEQ ID NO: 22 - protein, 48 aa, Homo sapiens; identical to SEQ ID NO: 5
  DCD-1L
  MOD_RES 6: ACETYLATION

SEQ ID NO: 23 - protein, 46 aa, Homo sapiens; identical to SEQ ID NO: 6
  SSL-46
  MOD_RES 6: ACETYLATION

SEQ ID NO: 24 - protein, 44 aa, Homo sapiens; identical to SEQ ID NO: 7
  LEK-44
  MOD_RES 3: ACETYLATION

SEQ ID NO: 25 - protein, 43 aa, Homo sapiens; identical to SEQ ID NO: 8
  LEK-43
  MOD_RES 3: ACETYLATION

SEQ ID NO: 26 - protein, 29 aa, Homo sapiens
  SSL-29
  MOD_RES 6: ACETYLATION
SSLLEKGLDGAKKAVGGLGKLGKDAVEDL

SEQ ID NO: 27 - protein, 25 aa, Homo sapiens
  SSL-25
  MOD_RES 6: ACETYLATION
SSLLEKGLDGAKKAVGGLGKLGKDA

SEQ ID NO: 28 - protein, 41 aa, Homo sapiens; identical to SEQ ID NO: 11
  LEK-41
  MOD_RES 3: ACETYLATION

SEQ ID NO: 29 - protein, 26 aa, Homo sapiens
  LEK-26
  MOD_RES 3: ACETYLATION
LEKGLDGAKKAVGGLGKLGKDAVEDL

SEQ ID NO: 30 - protein, 24 aa, Homo sapiens
  LEK-24
  MOD_RES 3: ACETYLATION
LEKGLDGAKKAVGGLGKLGKDAVE

SEQ ID NO: 31 - protein, 110 aa, Homo sapiens; identical to SEQ ID NO: 17
  Dermcidin
  MOD_RES 68: ACETYLATION